European Patent Application EP 4 321 180 A1, published February 14, 2024. Title: Antibody-drug conjugate comprising antibody binding to antibody against human CLDN18.2 and its use. Applicant: LEGOCHEM BIOSCIENCES, INC. The sequence listing filed with the application follows.

SEQUENCE LISTING (21 sequences)

SEQ ID NO: 1 - protein, 25 aa, Artificial Sequence
  PR002726 VH FR1
EVQLLESGGGLVQPGGSLRLSCAAS

SEQ ID NO: 2 - protein, 10 aa, Artificial Sequence
  PR002726 VH CDR1
GFTFSSFVMS

SEQ ID NO: 3 - protein, 14 aa, Artificial Sequence
  PR002726 VH FR2
WVRQAPGKGLEWVS

SEQ ID NO: 4 - protein, 17 aa, Artificial Sequence
  PR002726 VH CDR2
TISGSGRSTYYADSVKG

SEQ ID NO: 5 - protein, 32 aa, Artificial Sequence
  PR002726 VH FR3
RFTISRDNSKNTLHLQMNSLRAEDTAVYYCAK

SEQ ID NO: 6 - protein, 11 aa, Artificial Sequence
  PR002726 VH CDR3
DAAAAGTKFDY

SEQ ID NO: 7 - protein, 11 aa, Artificial Sequence
  PR002726 VH FR4
WGQGTLVTVSS

SEQ ID NO: 8 - protein, 23 aa, Artificial Sequence
  PR002726 VL FR1
EIVLTQSPATLSLSPGERATLSC

SEQ ID NO: 9 - protein, 11 aa, Artificial Sequence
  PR002726 VL CDR1
RASQSVSSYLA

SEQ ID NO: 10 - protein, 15 aa, Artificial Sequence
  PR002726 VL FR2
WYQQKPGQAPRLLIY

SEQ ID NO: 11 - protein, 7 aa, Artificial Sequence
  PR002726 VL CDR2
DASNRAT

SEQ ID NO: 12 - protein, 32 aa, Artificial Sequence
  PR002726 VL FR3
GIPARFSGSGSGTDFTLTISSLEPEDFAVYYC

SEQ ID NO: 13 - protein, 9 aa, Artificial Sequence
  PR002726 VL CDR3
QQRSNWPLT

SEQ ID NO: 14 - protein, 10 aa, Artificial Sequence
  PR002726 VL FR4
FGGGTKVEIK

SEQ ID NO: 15 - protein, 120 aa, Artificial Sequence
  PR002726 VH
EVQLLESGGGLVQPGGSLRLSCAASGFTFSSFVMSWVRQAPGKGLEWVSTISGSGRSTYYADSVKGRFTISRDNSKNTLHLQMNSLRAEDTAVYYCAKDAAAAGTKFDYWGQGTLVTVSS

SEQ ID NO: 16 - protein, 107 aa, Artificial Sequence
  PR002726 VL
EIVLTQSPATLSLSPGERATLSCRASQSVSSYLAWYQQKPGQAPRLLIYDASNRATGIPARFSGSGSGTDFTLTISSLEPEDFAVYYCQQRSNWPLTFGGGTKVEIK

SEQ ID NO: 17 - protein, 450 aa, Artificial Sequence
  PR002726 HC
EVQLLESGGGLVQPGGSLRLSCAASGFTFSSFVMSWVRQAPGKGLEWVSTISGSGRSTYYADSVKGRFTISRDNSKNTLHLQMNSLRAEDTAVYYCAKDAAAAGTKFDYWGQGTLVTVSSASTKGPSVFPLAPSSKSTSGGTAALGCLVKDYFPEPVTVSWNSGALTSGVHTFPAVLQSSGLYSLSSVVTVPSSSLGTQTYICNVNHKPSNTKVDKKVEPKSCDKTHTCPPCPAPELLGGPSVFLFPPKPKDTLMISRTPEVTCVVVDVSHEDPEVKFNWYVDGVEVHNAKTKPREEQYNSTYRVVSVLTVLHQDWLNGKEYKCKVSNKALPAPIEKTISKAKGQPREPQVYTLPPSREEMTKNQVSLTCLVKGFYPSDIAVEWESNGQPENNYKTTPPVLDSDGSFFLYSKLTVDKSRWQQGNVFSCSVMHEALHNHYTQKSLSLSPGK

SEQ ID NO: 18 - protein, 214 aa, Artificial Sequence
  PR002726 LC
EIVLTQSPATLSLSPGERATLSCRASQSVSSYLAWYQQKPGQAPRLLIYDASNRATGIPARFSGSGSGTDFTLTISSLEPEDFAVYYCQQRSNWPLTFGGGTKVEIKRTVAAPSVFIFPPSDEQLKSGTASVVCLLNNFYPREAKVQWKVDNALQSGNSQESVTEQDSKDSTYSLSSTLTLSKADYEKHKVYACEVTHQGLSSPVTKSFNRGEC

SEQ ID NO: 19 - protein, 11 aa, Artificial Sequence
  CaaX peptide
GGGGGGGCVIM

SEQ ID NO: 20 - protein, 21 aa, Artificial Sequence
  PR301839 VL FR4
FGGGTKVEIKGGGGGGGCVIM

SEQ ID NO: 21 - protein, 118 aa, Artificial Sequence
  PR301839 VL
EIVLTQSPATLSLSPGERATLSCRASQSVSSYLAWYQQKPGQAPRLLIYDASNRATGIPARFSGSGSGTDFTLTISSLEPEDFAVYYCQQRSNWPLTFGGGTKVEIKGGGGGGGCVIM